European Patent Application EP 4 233 912 A2, published August 30, 2023. Title: Compositions for use as a prophylactic agent to those at risk of infection of tuberculosis, or as secondary agents for treating infected tuberculosis patients. Applicant: Universidad de Zaragoza. The sequence listing filed with the application follows.

SEQUENCE LISTING (4 sequences)

SEQ ID NO: 1 - DNA, 1752 bp, Mycobacterium tuberculosis
  misc_feature 1..1752: note = wild-type fadD26 gene in Mt103
  source 1..1752: mol_type = other DNA
atgccggtgaccgaccgttcagtgccctctttgctgcaagagagggccgaccagcagcctgacagcactgcatatacgtacatcgactacggatccgaccccaagggatttgctgacagcttgacttggtcgcaggtctacagtcgtgcatgcatcattgctgaagaactcaagttatgcgggttacccggagatcgagtggcggttttagcgccacaaggactggaatatgtccttgcattcctgggcgcacttcaggctggatttatcgcggttccgctgtcaactccacagtatggcattcacgatgaccgcgtttctgcggtgttgcaggattccaagccggtagccattctcacgacttcgtccgtggtaggcgatgtaacgaaatacgcagccagccacgacgggcagcctgccccggtcgtagttgaggttgatctgcttgatttggactcgccgcgacagatgccggctttctctcgtcagcacaccggggcggcttatctccaatacacgtccggatcgacgcgtacgccggccggagtcattgtgtcgcacacgaatgtcattgccaatgtgacacaaagtatgtacggctatttcggcgatcccgcaaagattccgaccgggactgtggtgtcgtggctgcctttgtatcacgatatgggcctgattctcggaatttgcgcaccgctggtggcccgacgccgcgcgatgttgatgagcccaatgtcatttttgcgccgtccggcccgctggatgcaactgcttgccaccagcggccggtgcttttctgcggcaccgaatttcgccttcgagctggccgtgcgcagaacatctgaccaggacatggcggggctcgacctgcgcgacgtggtcggcatcgtcagtggcagtgagcgaatccatgtggcaaccgtgcggcggttcatcgagcggttcgcgccgtacaatctcagccccaccgcgatacggccgtcgtacgggctcgcggaagcgaccttatatgtggcagctcccgaagccggcgccgcgcccaagacggtccgttttgactacgagcagctgaccgccgggcaggctcggccctgcggaaccgatgggtcggtcggcaccgaactgatcagctacggctcccccgacccatcgtctgtgcgaatcgtcaacccggagaccatggttgagaatccgcctggagtggtcggtgagatctgggtgcatggcgaccacgtgactatggggtattggcagaagccgaagcagaccgcgcaggtcttcgacgccaagctggtcgatcccgcgccggcagccccggaggggccgtggctgcgcaccggcgacctgggcgtcatttccgatggtgagctgttcatcatgggccgcatcaaagacctgctcatcgtggacgggcgcaaccactaccccgacgacatcgaggcaacgatccaggagatcaccggtggacgggccgcggcgatcgcagtgcccgacgacatcaccgaacaactggtggcgatcatcgaattcaagcgacgcggtagtaccgccgaagaggtcatgctcaagctccgctcggtgaagcgtgaggtcacctccgcgatatcgaagtcacacagcctgcgggtggccgatctcgttctggtgtcacctggttcgattcccatcaccaccagcggcaagatccggcggtcagcctgcgtcgaacgctatcgcagcgacggcttcaagcggctggacgtagccgtatga

SEQ ID NO: 2 - DNA, 410 bp, Mycobacterium tuberculosis
  misc_feature 1..410: note = fadD26 in MTBVAC
  source 1..410: mol_type = other DNA
atgccggtgaccgaccgttcagtgccctctttgctgcaagagagggccgaccagcagcctgacagcactgcatatacgtacatcgactacggatccactagttctagagcaaccgtccgaaatattataaattatcgcacacataaaaacagtgctgttaatgtgtctattaaatcgattttttgttataacagacactgcttgtccgatatttgatttaggatacatttttatgagatcccccgggctgcaggaattcgatatcgaagtcacacagcctgcgggtggccgatctcgttctggtgtcacctggttcgattcccatcaccaccagcggcaagatccggcggtcagcctgcgtcgaacgctatcgcagcgacggcttcaagcggctggacgtagccgtatga

SEQ ID NO: 3 - DNA, 744 bp, Mycobacterium tuberculosis
  misc_feature 1..744: note = wild-type phoP gene in Mt103
  source 1..744: mol_type = other DNA
atgcggaaaggggttgatctcgtgacggcgggaaccccaggcgaaaacaccacaccggaggctcgtgtcctcgtggtcgatgatgaggccaacatcgttgaactgctgtcggtgagcctcaagttccagggctttgaagtctacaccgcgaccaacggggcacaggcgctggatcgggcccgggaaacccggccggacgcggtgatcctcgatgtgatgatgcccgggatggacggctttggggtgctgcgccggctgcgcgccgacggcatcgatgccccggcgttgttcctgacggcccgtgactcgctacaggacaagatcgcgggtctgaccctgggtggtgacgactatgtgacaaagcccttcagtttggaggaggtcgtggccaggctgcgggtcatcctgcgacgcgcgggcaagggcaacaaggaaccacgtaatgttcgactgacgttcgccgatatcgagctcgacgaggagacccacgaagtgtggaaggcgggccaaccggtgtcgctgtcgcccaccgaattcaccctgctgcgctatttcgtgatcaacgcgggcaccgtgctgagcaagcctaagattctcgaccacgtttggcgctacgacttcggtggtgatgtcaacgtcgtcgagtcctacgtgtcgtatctgcgccgcaagatcgacactggggagaagcggctgctgcacacgctgcgcggggtgggctacgtactgcgggagcctcgatga

SEQ ID NO: 4 - DNA, 819 bp, Mycobacterium tuberculosis
  misc_feature 1..819: note = phoP in MTBVAC
  source 1..819: mol_type = other DNA
atgcggaaaggggttgatctcgtgacggcgggaaccccaggcgaaaacaccacaccggaggctcgtgtcctcgtggtcgatgatgaggccaacatcgttgaactgctgtcggtgagcctcaagttccagggctttgaagtctacaccgcgaccaacggggcacaggcgctggatcgggcccgggaaacccggccggacgcggtgatcctcgatgtgatgatgcccgggatggacggctttggggtgctgcgccggctgcgcgccgacggcatcgatgccccggcgttgttcctgacggcccgtgactcgctacaggacaagatcgcgggtctgaccctgggtggtgacgactatgtgacaaagcccttcagtttggaggaggtcgtggccaggctgcgggtcatcctgcgacgcgcgggcaagggcaacaaggaaccacgtaatgttcgactgacgttcgccgatatcgaattcctgcagcccgggggatctcataaaaatgtatcctaaatcaaatatcggacaagcagtgtctgttataacaaaaaatcgatttaatagacacattaacagcactgtttttatgtgtgcgataatttataatatttcggacggttgctctagaactagtggatcaacgcgggcaccgtgctgagcaagcctaagattctcgaccacgtttggcgctacgacttcggtggtgatgtcaacgtcgtcgagtcctacgtgtcgtatctgcgccgcaagatcgacactggggagaagcggctgctgcacacgctgcgcggggtgggctacgtactgcgggagcctcgatga